European Patent Specification EP 4 176 089 B1, published September 10, 2025. Title: RAPID DETECTION KIT FOR HUMAN PATHOGENIC CORONAVIRUSES : BETACORONAVIRUS GROUP B/C AND SARS-CoV-2. Applicant: INSTITUT PASTEUR. The sequence listing filed with the application follows.

SEQUENCE LISTING (226 sequences)

SEQ ID NO: 1 - DNA, 1260 bp, SARS-CoV-2
atgtctgataatggaccccaaaatcagcgaaatgcaccccgcattacgtttggtggaccctcagattcaactggcagtaaccagaatggagaacgcagtggggcgcgatcaaaacaacgtcggccccaaggtttacccaataatactgcgtcttggttcaccgctctcactcaacatggcaaggaagaccttaaattccctcgaggacaaggcgttccaattaacaccaatagcagtccagatgaccaaattggctactaccgaagagctaccagacgaattcgtggtggtgacggtaaaatgaaagatctcagtccaagatggtatttctactacctaggaactgggccagaagctggacttccctatggtgctaacaaagacggcatcatatgggttgcaactgagggagccttgaatacaccaaaagatcacattggcacccgcaatcctgctaacaatgctgcaatcgtgctacaacttcctcaaggaacaacattgccaaaaggcttctacgcagaagggagcagaggcggcagtcaagcctcttctcgttcctcatcacgtagtcgcaacagttcaagaaattcaactccaggcagcagtaggggaacttctcctgctagaatggctggcaatggcggtgatgctgctcttgctttgctgctgcttgacagattgaaccagcttgagagcaaaatgtctggtaaaggccaacaacaacaaggccaaactgtcactaagaaatctgctgctgaggcttctaagaagcctcggcaaaaacgtactgccactaaagcatacaatgtaacacaagctttcggcagacgtggtccagaacaaacccaaggaaattttggggaccaggaactaatcagacaaggaactgattacaaacattggccgcaaattgcacaatttgcccccagcgcttcagcgttcttcggaatgtcgcgcattggcatggaagtcacaccttcgggaacgtggttgacctacacaggtgccatcaaattggatgacaaagatccaaatttcaaagatcaagtcattttgctgaataagcatattgacgcatacaaaacattcccaccaacagagcctaaaaaggacaaaaagaagaaggctgatgaaactcaagccttaccgcagagacagaagaaacagcaaactgtgactcttcttcctgctgcagatttggatgatttctccaaacaattgcaacaatccatgagcagtgctgactcaactcaggcctaa

SEQ ID NO: 2 - DNA, 2795 bp, SARS-CoV-2
tcagctgatgcacaatcgtttttaaacgggtttgcggtgtaagtgcagcccgtcttacaccgtgcggcacaggcactagtactgatgtcgtatacagggcttttgacatctacaatgataaagtagctggttttgctaaattcctaaaaactaattgttgtcgcttccaagaaaaggacgaagatgacaatttaattgattcttactttgtagttaagagacacactttctctaactaccaacatgaagaaacaatttataatttacttaaggattgtccagctgttgctaaacatgacttctttaagtttagaatagacggtgacatggtaccacatatatcacgtcaacgtcttactaaatacacaatggcagacctcgtctatgctttaaggcattttgatgaaggtaattgtgacacattaaaagaaatacttgtcacatacaattgttgtgatgatgattatttcaataaaaaggactggtatgattttgtagaaaacccagatatattacgcgtatacgccaacttaggtgaacgtgtacgccaagctttgttaaaaacagtacaattctgtgatgccatgcgaaatgctggtattgttggtgtactgacattagataatcaagatctcaatggtaactggtatgatttcggtgatttcatacaaaccacgccaggtagtggagttcctgttgtagattcttattattcattgttaatgcctatattaaccttgaccagggctttaactgcagagtcacatgttgacactgacttaacaaagccttacattaagtgggatttgttaaaatatgacttcacggaagagaggttaaaactctttgaccgttattttaaatattgggatcagacataccacccaaattgtgttaactgtttggatgacagatgcattctgcattgtgcaaactttaatgttttattctctacagtgttcccacctacaagttttggaccactagtgagaaaaatatttgttgatggtgttccatttgtagtttcaactggataccacttcagagagctaggtgttgtacataatcaggatgtaaacttacatagctctagacttagttttaaggaattacttgtgtatgctgctgaccctgctatgcacgctgcttctggtaatctattactagataaacgcactacgtgcttttcagtagctgcacttactaacaatgttgcttttcaaactgtcaaacccggtaattttaacaaagacttctatgactttgctgtgtctaagggtttctttaaggaaggaagttctgttgaattaaaacacttcttctttgctcaggatggtaatgctgctatcagcgattatgactactatcgttataatctaccaacaatgtgtgatatcagacaactactatttgtagttgaagttgttgataagtactttgattgttacgatggtggctgtattaatgctaaccaagtcatcgtcaacaacctagacaaatcagctggttttccatttaataaatggggtaaggctagactttattatgattcaatgagttatgaggatcaagatgcacttttcgcatatacaaaacgtaatgtcatccctactataactcaaatgaatcttaagtatgccattagtgcaaagaatagagctcgcaccgtagctggtgtctctatctgtagtactatgaccaatagacagtttcatcaaaaattattgaaatcaatagccgccactagaggagctactgtagtaattggaacaagcaaattctatggtggttggcacaacatgttaaaaactgtttatagtgatgtagaaaaccctcaccttatgggttgggattatcctaaatgtgatagagccatgcctaacatgcttagaattatggcctcacttgttcttgctcgcaaacatacaacgtgttgtagcttgtcacaccgtttctatagattagctaatgagtgtgctcaagtattgagtgaaatggtcatgtgtggcggttcactatatgttaaaccaggtggaacctcatcaggagatgccacaactgcttatgctaatagtgtttttaacatttgtcaagctgtcacggccaatgttaatgcacttttatctactgatggtaacaaaattgccgataagtatgtccgcaatttacaacacagactttatgagtgtctctatagaaatagagatgttgacacagactttgtgaatgagttttacgcatatttgcgtaaacatttctcaatgatgatactctctgacgatgctgttgtgtgtttcaatagcacttatgcatctcaaggtctagtggctagcataaagaactttaagtcagttctttattatcaaaacaatgtttttatgtctgaagcaaaatgttggactgagactgaccttactaaaggacctcatgaattttgctctcaacatacaatgctagttaaacagggtgatgattatgtgtaccttccttacccagatccatcaagaatcctaggggccggctgttttgtagatgatatcgtaaaaacagatggtacacttatgattgaacggttcgtgtctttagctatagatgcttacccacttactaaacatcctaatcaggagtatgctgatgtctttcatttgtacttacaatacataagaaagctacatgatgagttaacaggacacatgttagacatgtattctgttatgcttactaatgataacacttcaaggtattgggaacctgagttttatgaggctatgtacacaccgcatacagtcttacag

SEQ ID NO: 3 - DNA, 18 bp, artificial sequence
  synthetic oligonucleotide
tcctgctaacaatgctgc

SEQ ID NO: 4 - DNA, 20 bp, artificial sequence
  synthetic oligonucleotide
tctcaagctggttcaatctg

SEQ ID NO: 5 - DNA, 40 bp, artificial sequence
  synthetic oligonucleotide
aacgagaagaggcttgactgctcaaggaacaacattgcca

SEQ ID NO: 6 - DNA, 40 bp, artificial sequence
  synthetic oligonucleotide
ctcatcacgtagtcgcaacagtattgccagccattctagc

SEQ ID NO: 7 - DNA, 19 bp, artificial sequence
  synthetic oligonucleotide
ccttctgcgtagaagcctt

SEQ ID NO: 8 - DNA, 19 bp, artificial sequence
  synthetic oligonucleotide
aattcaactccaggcagca

SEQ ID NO: 9 - DNA, 19 bp, artificial sequence
  synthetic oligonucleotide
tcaaggaacaacattgcca

SEQ ID NO: 10 - DNA, 21 bp, artificial sequence
  synthetic oligonucleotide
aacgagaagaggcttgactgc

SEQ ID NO: 11 - DNA, 18 bp, artificial sequence
  synthetic oligonucleotide
attgccagccattctagc

SEQ ID NO: 12 - DNA, 22 bp, artificial sequence
  synthetic oligonucleotide
ctcatcacgtagtcgcaacagt

SEQ ID NO: 13 - DNA, 154 bp, artificial sequence
  synthetic oligonucleotide
tcaaggaacaacattgccaaaaggcttctacgcagaagggagcagaggcggcagtcaagcctcttctcgttcctcatcacgtagtcgcaacagttcaagaaattcaactccaggcagcagtaggggaacttctcctgctagaatggctggcaat

SEQ ID NO: 14 - DNA, 19 bp, artificial sequence
  synthetic oligonucleotide
tcaaggaacaacattgcca

SEQ ID NO: 15 - DNA, 20 bp, artificial sequence
  synthetic oligonucleotide
cttcttagaagcctcagcag

SEQ ID NO: 16 - DNA, 38 bp, artificial sequence
  synthetic oligonucleotide
gccagccattctagcaggagcacgtagtcgcaacagtt

SEQ ID NO: 17 - DNA, 38 bp, artificial sequence
  synthetic oligonucleotide
aatggcggtgatgctgcttctcaagctggttcaatctg

SEQ ID NO: 18 - DNA, 19 bp, artificial sequence
  synthetic oligonucleotide
tgctgcctggagttgaatt

SEQ ID NO: 19 - DNA, 18 bp, artificial sequence
  synthetic oligonucleotide
ttgctttgctgctgcttg

SEQ ID NO: 20 - DNA, 18 bp, artificial sequence
  synthetic oligonucleotide
cacgtagtcgcaacagtt

SEQ ID NO: 21 - DNA, 20 bp, artificial sequence
  synthetic oligonucleotide
gccagccattctagcaggag

SEQ ID NO: 22 - DNA, 20 bp, artificial sequence
  synthetic oligonucleotide
tctcaagctggttcaatctg

SEQ ID NO: 23 - DNA, 18 bp, artificial sequence
  synthetic oligonucleotide
aatggcggtgatgctgct

SEQ ID NO: 24 - DNA, 132 bp, artificial sequence
  synthetic oligonucleotide
cacgtagtcgcaacagttcaagaaattcaactccaggcagcagtaggggaacttctcctgctagaatggctggcaatggcggtgatgctgctcttgctttgctgctgcttgacagattgaaccagcttgaga

SEQ ID NO: 25 - DNA, 19 bp, artificial sequence
  synthetic oligonucleotide
tcaaggaacaacattgcca

SEQ ID NO: 26 - DNA, 20 bp, artificial sequence
  synthetic oligonucleotide
cttcttagaagcctcagcag

SEQ ID NO: 27 - DNA, 38 bp, artificial sequence
  synthetic oligonucleotide
gccagccattctagcaggagcgtagtcgcaacagttca

SEQ ID NO: 28 - DNA, 38 bp, artificial sequence; identical to SEQ ID NO: 17
  synthetic oligonucleotide

SEQ ID NO: 29 - DNA, 19 bp, artificial sequence
  synthetic oligonucleotide
tgctgcctggagttgaatt

SEQ ID NO: 30 - DNA, 18 bp, artificial sequence
  synthetic oligonucleotide
ttgctttgctgctgcttg

SEQ ID NO: 31 - DNA, 18 bp, artificial sequence
  synthetic oligonucleotide
cgtagtcgcaacagttca

SEQ ID NO: 32 - DNA, 20 bp, artificial sequence
  synthetic oligonucleotide
gccagccattctagcaggag

SEQ ID NO: 33 - DNA, 20 bp, artificial sequence
  synthetic oligonucleotide
tctcaagctggttcaatctg

SEQ ID NO: 34 - DNA, 18 bp, artificial sequence
  synthetic oligonucleotide
aatggcggtgatgctgct

SEQ ID NO: 35 - DNA, 130 bp, artificial sequence
  synthetic oligonucleotide
cgtagtcgcaacagttcaagaaattcaactccaggcagcagtaggggaacttctcctgctagaatggctggcaatggcggtgatgctgctcttgctttgctgctgcttgacagattgaaccagcttgaga

SEQ ID NO: 36 - DNA, 20 bp, artificial sequence
  synthetic oligonucleotide
aatcgtgctacaacttcctc

SEQ ID NO: 37 - DNA, 21 bp, artificial sequence
  synthetic oligonucleotide
ctcagcagcagatttcttagt

SEQ ID NO: 38 - DNA, 38 bp, artificial sequence
  synthetic oligonucleotide
cctactgctgcctggagttgagtcaagcctcttctcgt

SEQ ID NO: 39 - DNA, 39 bp, artificial sequence
  synthetic oligonucleotide
ctcctgctagaatggctggctcaatctgtcaagcagcag

SEQ ID NO: 40 - DNA, 19 bp, artificial sequence
  synthetic oligonucleotide
ttgcgactacgtgatgagg

SEQ ID NO: 41 - DNA, 18 bp, artificial sequence
  synthetic oligonucleotide
ggtgatgctgctcttgct

SEQ ID NO: 42 - DNA, 18 bp, artificial sequence
  synthetic oligonucleotide
agtcaagcctcttctcgt

SEQ ID NO: 43 - DNA, 20 bp, artificial sequence
  synthetic oligonucleotide
cctactgctgcctggagttg

SEQ ID NO: 44 - DNA, 19 bp, artificial sequence
  synthetic oligonucleotide
tcaatctgtcaagcagcag

SEQ ID NO: 45 - DNA, 20 bp, artificial sequence
  synthetic oligonucleotide
ctcctgctagaatggctggc

SEQ ID NO: 46 - DNA, 145 bp, artificial sequence
  synthetic oligonucleotide
agtcaagcctcttctcgttcctcatcacgtagtcgcaacagttcaagaaattcaactccaggcagcagtaggggaacttctcctgctagaatggctggcaatggcggtgatgctgctcttgctttgctgctgcttgacagattga

SEQ ID NO: 47 - DNA, 20 bp, artificial sequence
  synthetic oligonucleotide
tcaaggaacaacattgccaa

SEQ ID NO: 48 - DNA, 20 bp, artificial sequence
  synthetic oligonucleotide
cttcttagaagcctcagcag

SEQ ID NO: 49 - DNA, 40 bp, artificial sequence
  synthetic oligonucleotide
gccagccattctagcaggaggtagtcgcaacagttcaaga

SEQ ID NO: 50 - DNA, 38 bp, artificial sequence; identical to SEQ ID NO: 17
  synthetic oligonucleotide

SEQ ID NO: 51 - DNA, 19 bp, artificial sequence
  synthetic oligonucleotide
tgctgcctggagttgaatt

SEQ ID NO: 52 - DNA, 18 bp, artificial sequence
  synthetic oligonucleotide
ttgctttgctgctgcttg

SEQ ID NO: 53 - DNA, 20 bp, artificial sequence
  synthetic oligonucleotide
gtagtcgcaacagttcaaga

SEQ ID NO: 54 - DNA, 20 bp, artificial sequence
  synthetic oligonucleotide
gccagccattctagcaggag

SEQ ID NO: 55 - DNA, 20 bp, artificial sequence
  synthetic oligonucleotide
tctcaagctggttcaatctg

SEQ ID NO: 56 - DNA, 18 bp, artificial sequence
  synthetic oligonucleotide
aatggcggtgatgctgct

SEQ ID NO: 57 - DNA, 129 bp, artificial sequence
  synthetic oligonucleotide
gtagtcgcaacagttcaagaaattcaactccaggcagcagtaggggaacttctcctgctagaatggctggcaatggcggtgatgctgctcttgctttgctgctgcttgacagattgaaccagcttgaga

SEQ ID NO: 58 - DNA, 18 bp, artificial sequence
  synthetic oligonucleotide
agtcaagcctcttctcgt

SEQ ID NO: 59 - DNA, 18 bp, artificial sequence
  synthetic oligonucleotide
tgccgaggcttcttagaa

SEQ ID NO: 60 - DNA, 36 bp, artificial sequence
  synthetic oligonucleotide
agcagcatcaccgccattaattcaactccaggcagc

SEQ ID NO: 61 - DNA, 39 bp, artificial sequence
  synthetic oligonucleotide
gctttgctgctgcttgacagttgttggcctttaccagac

SEQ ID NO: 62 - DNA, 19 bp, artificial sequence
  synthetic oligonucleotide
ccagccattctagcaggag

SEQ ID NO: 63 - DNA, 20 bp, artificial sequence
  synthetic oligonucleotide
attgaaccagcttgagagca

SEQ ID NO: 64 - DNA, 18 bp, artificial sequence
  synthetic oligonucleotide
aattcaactccaggcagc

SEQ ID NO: 65 - DNA, 18 bp, artificial sequence
  synthetic oligonucleotide
agcagcatcaccgccatt

SEQ ID NO: 66 - DNA, 19 bp, artificial sequence
  synthetic oligonucleotide
ttgttggcctttaccagac

SEQ ID NO: 67 - DNA, 20 bp, artificial sequence
  synthetic oligonucleotide
gctttgctgctgcttgacag

SEQ ID NO: 68 - DNA, 135 bp, artificial sequence
  synthetic oligonucleotide
aattcaactccaggcagcagtaggggaacttctcctgctagaatggctggcaatggcggtgatgctgctcttgctttgctgctgcttgacagattgaaccagcttgagagcaaaatgtctggtaaaggccaacaa

SEQ ID NO: 69 - DNA, 19 bp, artificial sequence
  synthetic oligonucleotide
ggcagtaaccagaatggag

SEQ ID NO: 70 - DNA, 22 bp, artificial sequence
  synthetic oligonucleotide
aataccatcttggactgagatc

SEQ ID NO: 71 - DNA, 38 bp, artificial sequence
  synthetic oligonucleotide
ttggaacgccttgtcctcgatactgcgtcttggttcac

SEQ ID NO: 72 - DNA, 40 bp, artificial sequence
  synthetic oligonucleotide
accaatagcagtccagatgacccgtcaccaccacgaattc

SEQ ID NO: 73 - DNA, 20 bp, artificial sequence
  synthetic oligonucleotide
ttccttgccatgttgagtga

SEQ ID NO: 74 - DNA, 21 bp, artificial sequence
  synthetic oligonucleotide
aattggctactaccgaagagc

SEQ ID NO: 75 - DNA, 19 bp, artificial sequence
  synthetic oligonucleotide
atactgcgtcttggttcac

SEQ ID NO: 76 - DNA, 19 bp, artificial sequence
  synthetic oligonucleotide
ttggaacgccttgtcctcg

SEQ ID NO: 77 - DNA, 18 bp, artificial sequence
  synthetic oligonucleotide
cgtcaccaccacgaattc

SEQ ID NO: 78 - DNA, 22 bp, artificial sequence
  synthetic oligonucleotide
accaatagcagtccagatgacc

SEQ ID NO: 79 - DNA, 153 bp, artificial sequence
  synthetic oligonucleotide
atactgcgtcttggttcaccgctctcactcaacatggcaaggaagaccttaaattccctcgaggacaaggcgttccaattaacaccaatagcagtccagatgaccaaattggctactaccgaagagctaccagacgaattcgtggtggtgacg

SEQ ID NO: 80 - DNA, 20 bp, artificial sequence
  synthetic oligonucleotide
caaggcgttccaattaacac

SEQ ID NO: 81 - DNA, 18 bp, artificial sequence
  synthetic oligonucleotide
gcagcattgttagcagga

SEQ ID NO: 82 - DNA, 40 bp, artificial sequence
  synthetic oligonucleotide
accgtcaccaccacgaattccaatagcagtccagatgacc

SEQ ID NO: 83 - DNA, 38 bp, artificial sequence
  synthetic oligonucleotide
ctaggaactgggccagaagcacccatatgatgccgtct

SEQ ID NO: 84 - DNA, 21 bp, artificial sequence
  synthetic oligonucleotide
gctcttcggtagtagccaatt

SEQ ID NO: 85 - DNA, 22 bp, artificial sequence
  synthetic oligonucleotide
gacttccctatggtgctaacaa

SEQ ID NO: 86 - DNA, 20 bp, artificial sequence
  synthetic oligonucleotide
caatagcagtccagatgacc

SEQ ID NO: 87 - DNA, 20 bp, artificial sequence
  synthetic oligonucleotide
accgtcaccaccacgaattc

SEQ ID NO: 88 - DNA, 18 bp, artificial sequence
  synthetic oligonucleotide
acccatatgatgccgtct

SEQ ID NO: 89 - DNA, 20 bp, artificial sequence
  synthetic oligonucleotide
ctaggaactgggccagaagc

SEQ ID NO: 90 - DNA, 171 bp, artificial sequence
  synthetic oligonucleotide
caatagcagtccagatgaccaaattggctactaccgaagagctaccagacgaattcgtggtggtgacggtaaaatgaaagatctcagtccaagatggtatttctactacctaggaactgggccagaagctggacttccctatggtgctaacaaagacggcatcatatgggt

SEQ ID NO: 91 - DNA, 19 bp, artificial sequence
  synthetic oligonucleotide
tcaacatggcaaggaagac

SEQ ID NO: 92 - DNA, 18 bp, artificial sequence
  synthetic oligonucleotide
gcagcattgttagcagga

SEQ ID NO: 93 - DNA, 41 bp, artificial sequence
  synthetic oligonucleotide
accgtcaccaccacgaattcttaacaccaatagcagtccag

SEQ ID NO: 94 - DNA, 38 bp, artificial sequence; identical to SEQ ID NO: 83
  synthetic oligonucleotide

SEQ ID NO: 95 - DNA, 21 bp, artificial sequence
  synthetic oligonucleotide
gctcttcggtagtagccaatt

SEQ ID NO: 96 - DNA, 22 bp, artificial sequence
  synthetic oligonucleotide
gacttccctatggtgctaacaa

SEQ ID NO: 97 - DNA, 21 bp, artificial sequence
  synthetic oligonucleotide
ttaacaccaatagcagtccag

SEQ ID NO: 98 - DNA, 20 bp, artificial sequence
  synthetic oligonucleotide
accgtcaccaccacgaattc

SEQ ID NO: 99 - DNA, 18 bp, artificial sequence
  synthetic oligonucleotide
acccatatgatgccgtct

SEQ ID NO: 100 - DNA, 20 bp, artificial sequence
  synthetic oligonucleotide
ctaggaactgggccagaagc

SEQ ID NO: 101 - DNA, 178 bp, artificial sequence
  synthetic oligonucleotide
ttaacaccaatagcagtccagatgaccaaattggctactaccgaagagctaccagacgaattcgtggtggtgacggtaaaatgaaagatctcagtccaagatggtatttctactacctaggaactgggccagaagctggacttccctatggtgctaacaaagacggcatcatatgggt

SEQ ID NO: 102 - DNA, 19 bp, artificial sequence
  synthetic oligonucleotide
tcaacatggcaaggaagac

SEQ ID NO: 103 - DNA, 18 bp, artificial sequence
  synthetic oligonucleotide
gcagcattgttagcagga

SEQ ID NO: 104 - DNA, 40 bp, artificial sequence
  synthetic oligonucleotide
accgtcaccaccacgaattcccaatagcagtccagatgac

SEQ ID NO: 105 - DNA, 38 bp, artificial sequence; identical to SEQ ID NO: 83
  synthetic oligonucleotide

SEQ ID NO: 106 - DNA, 21 bp, artificial sequence
  synthetic oligonucleotide
gctcttcggtagtagccaatt

SEQ ID NO: 107 - DNA, 22 bp, artificial sequence
  synthetic oligonucleotide
gacttccctatggtgctaacaa

SEQ ID NO: 108 - DNA, 20 bp, artificial sequence
  synthetic oligonucleotide
ccaatagcagtccagatgac

SEQ ID NO: 109 - DNA, 20 bp, artificial sequence
  synthetic oligonucleotide
accgtcaccaccacgaattc

SEQ ID NO: 110 - DNA, 18 bp, artificial sequence
  synthetic oligonucleotide
acccatatgatgccgtct

SEQ ID NO: 111 - DNA, 20 bp, artificial sequence
  synthetic oligonucleotide
ctaggaactgggccagaagc

SEQ ID NO: 112 - DNA, 172 bp, artificial sequence
  synthetic oligonucleotide
ccaatagcagtccagatgaccaaattggctactaccgaagagctaccagacgaattcgtggtggtgacggtaaaatgaaagatctcagtccaagatggtatttctactacctaggaactgggccagaagctggacttccctatggtgctaacaaagacggcatcatatgggt

SEQ ID NO: 113 - DNA, 20 bp, artificial sequence
  synthetic oligonucleotide
caaggcgttccaattaacac

SEQ ID NO: 114 - DNA, 18 bp, artificial sequence
  synthetic oligonucleotide
gcagcattgttagcagga

SEQ ID NO: 115 - DNA, 39 bp, artificial sequence
  synthetic oligonucleotide
accgtcaccaccacgaattcatagcagtccagatgacca

SEQ ID NO: 116 - DNA, 38 bp, artificial sequence; identical to SEQ ID NO: 83
  synthetic oligonucleotide

SEQ ID NO: 117 - DNA, 21 bp, artificial sequence
  synthetic oligonucleotide
gctcttcggtagtagccaatt

SEQ ID NO: 118 - DNA, 22 bp, artificial sequence
  synthetic oligonucleotide
gacttccctatggtgctaacaa

SEQ ID NO: 119 - DNA, 19 bp, artificial sequence
  synthetic oligonucleotide
atagcagtccagatgacca

SEQ ID NO: 120 - DNA, 20 bp, artificial sequence
  synthetic oligonucleotide
accgtcaccaccacgaattc

SEQ ID NO: 121 - DNA, 18 bp, artificial sequence
  synthetic oligonucleotide
acccatatgatgccgtct

SEQ ID NO: 122 - DNA, 20 bp, artificial sequence
  synthetic oligonucleotide
ctaggaactgggccagaagc

SEQ ID NO: 123 - DNA, 169 bp, artificial sequence
  synthetic oligonucleotide
atagcagtccagatgaccaaattggctactaccgaagagctaccagacgaattcgtggtggtgacggtaaaatgaaagatctcagtccaagatggtatttctactacctaggaactgggccagaagctggacttccctatggtgctaacaaagacggcatcatatgggt

SEQ ID NO: 124 - DNA, 18 bp, artificial sequence
  synthetic oligonucleotide
tatggtggttggcacaac

SEQ ID NO: 125 - DNA, 18 bp, artificial sequence
  synthetic oligonucleotide
tgtggcatctcctgatga

SEQ ID NO: 126 - DNA, 43 bp, artificial sequence
  synthetic oligonucleotide
tgcgagcaagaacaagtgaggtgggttgggattatcctaaatg

SEQ ID NO: 127 - DNA, 42 bp, artificial sequence
  synthetic oligonucleotide
tgttgtagcttgtcacaccgttccacacatgaccatttcact

SEQ ID NO: 128 - DNA, 20 bp, artificial sequence
  synthetic oligonucleotide
taagcatgttaggcatggct

SEQ ID NO: 129 - DNA, 21 bp, artificial sequence
  synthetic oligonucleotide
agctaatgagtgtgctcaagt

SEQ ID NO: 130 - DNA, 22 bp, artificial sequence
  synthetic oligonucleotide
tgggttgggattatcctaaatg

SEQ ID NO: 131 - DNA, 21 bp, artificial sequence
  synthetic oligonucleotide
tgcgagcaagaacaagtgagg

SEQ ID NO: 132 - DNA, 20 bp, artificial sequence
  synthetic oligonucleotide
ccacacatgaccatttcact

SEQ ID NO: 133 - DNA, 22 bp, artificial sequence
  synthetic oligonucleotide
tgttgtagcttgtcacaccgtt

SEQ ID NO: 134 - DNA, 166 bp, artificial sequence
  synthetic oligonucleotide
tgggttgggattatcctaaatgtgatagagccatgcctaacatgcttagaattatggcctcacttgttcttgctcgcaaacatacaacgtgttgtagcttgtcacaccgtttctatagattagctaatgagtgtgctcaagtattgagtgaaatggtcatgtgtgg

SEQ ID NO: 135 - DNA, 18 bp, artificial sequence
  synthetic oligonucleotide
tatggtggttggcacaac

SEQ ID NO: 136 - DNA, 18 bp, artificial sequence
  synthetic oligonucleotide
tgtggcatctcctgatga

SEQ ID NO: 137 - DNA, 43 bp, artificial sequence
  synthetic oligonucleotide
tgcgagcaagaacaagtgagggggttgggattatcctaaatgt

SEQ ID NO: 138 - DNA, 42 bp, artificial sequence; identical to SEQ ID NO: 127
  synthetic oligonucleotide

SEQ ID NO: 139 - DNA, 20 bp, artificial sequence
  synthetic oligonucleotide
taagcatgttaggcatggct

SEQ ID NO: 140 - DNA, 21 bp, artificial sequence
  synthetic oligonucleotide
agctaatgagtgtgctcaagt

SEQ ID NO: 141 - DNA, 22 bp, artificial sequence
  synthetic oligonucleotide
gggttgggattatcctaaatgt

SEQ ID NO: 142 - DNA, 21 bp, artificial sequence
  synthetic oligonucleotide
tgcgagcaagaacaagtgagg

SEQ ID NO: 143 - DNA, 20 bp, artificial sequence
  synthetic oligonucleotide
ccacacatgaccatttcact

SEQ ID NO: 144 - DNA, 22 bp, artificial sequence
  synthetic oligonucleotide
tgttgtagcttgtcacaccgtt

SEQ ID NO: 145 - DNA, 165 bp, artificial sequence
  synthetic oligonucleotide
gggttgggattatcctaaatgtgatagagccatgcctaacatgcttagaattatggcctcacttgttcttgctcgcaaacatacaacgtgttgtagcttgtcacaccgtttctatagattagctaatgagtgtgctcaagtattgagtgaaatggtcatgtgtgg

SEQ ID NO: 146 - DNA, 18 bp, artificial sequence
  synthetic oligonucleotide
gcctcacttgttcttgct

SEQ ID NO: 147 - DNA, 20 bp, artificial sequence
  synthetic oligonucleotide
cggacatacttatcggcaat

SEQ ID NO: 148 - DNA, 38 bp, artificial sequence
  synthetic oligonucleotide
aaccgccacacatgaccattttgtagcttgtcacaccg

SEQ ID NO: 149 - DNA, 39 bp, artificial sequence
  synthetic oligonucleotide
aggtggaacctcatcaggagaccgtgacagcttgacaaa

SEQ ID NO: 150 - DNA, 22 bp, artificial sequence
  synthetic oligonucleotide
tcactcaatacttgagcacact

SEQ ID NO: 151 - DNA, 20 bp, artificial sequence
  synthetic oligonucleotide
tgccacaactgcttatgcta

SEQ ID NO: 152 - DNA, 18 bp, artificial sequence
  synthetic oligonucleotide
ttgtagcttgtcacaccg

SEQ ID NO: 153 - DNA, 20 bp, artificial sequence
  synthetic oligonucleotide
aaccgccacacatgaccatt

SEQ ID NO: 154 - DNA, 18 bp, artificial sequence
  synthetic oligonucleotide
ccgtgacagcttgacaaa

SEQ ID NO: 155 - DNA, 21 bp, artificial sequence
  synthetic oligonucleotide
aggtggaacctcatcaggaga

SEQ ID NO: 156 - DNA, 170 bp, artificial sequence
  synthetic oligonucleotide
ttgtagcttgtcacaccgtttctatagattagctaatgagtgtgctcaagtattgagtgaaatggtcatgtgtggcggttcactatatgttaaaccaggtggaacctcatcaggagatgccacaactgcttatgctaatagtgtttttaacatttgtcaagctgtcacgg

SEQ ID NO: 157 - DNA, 18 bp, artificial sequence
  synthetic oligonucleotide
gcctcacttgttcttgct

SEQ ID NO: 158 - DNA, 20 bp, artificial sequence
  synthetic oligonucleotide
cggacatacttatcggcaat

SEQ ID NO: 159 - DNA, 39 bp, artificial sequence
  synthetic oligonucleotide
ccgccacacatgaccatttctgttgtagcttgtcacacc

SEQ ID NO: 160 - DNA, 39 bp, artificial sequence; identical to SEQ ID NO: 149
  synthetic oligonucleotide

SEQ ID NO: 161 - DNA, 22 bp, artificial sequence
  synthetic oligonucleotide
actcaatacttgagcacactca

SEQ ID NO: 162 - DNA, 20 bp, artificial sequence
  synthetic oligonucleotide
tgccacaactgcttatgcta

SEQ ID NO: 163 - DNA, 19 bp, artificial sequence
  synthetic oligonucleotide
tgttgtagcttgtcacacc

SEQ ID NO: 164 - DNA, 20 bp, artificial sequence
  synthetic oligonucleotide
ccgccacacatgaccatttc

SEQ ID NO: 165 - DNA, 18 bp, artificial sequence
  synthetic oligonucleotide
ccgtgacagcttgacaaa

SEQ ID NO: 166 - DNA, 21 bp, artificial sequence
  synthetic oligonucleotide
aggtggaacctcatcaggaga

SEQ ID NO: 167 - DNA, 172 bp, artificial sequence
  synthetic oligonucleotide
tgttgtagcttgtcacaccgtttctatagattagctaatgagtgtgctcaagtattgagtgaaatggtcatgtgtggcggttcactatatgttaaaccaggtggaacctcatcaggagatgccacaactgcttatgctaatagtgtttttaacatttgtcaagctgtcacgg

SEQ ID NO: 168 - DNA, 21 bp, artificial sequence
  synthetic oligonucleotide
ccttatgggttgggattatcc

SEQ ID NO: 169 - DNA, 19 bp, artificial sequence
  synthetic oligonucleotide
attaacattggccgtgaca

SEQ ID NO: 170 - DNA, 43 bp, artificial sequence
  synthetic oligonucleotide
aacggtgtgacaagctacaacagcttagaattatggcctcact

SEQ ID NO: 171 - DNA, 39 bp, artificial sequence
  synthetic oligonucleotide
gtcatgtgtggcggttcactaaagcagttgtggcatctc

SEQ ID NO: 172 - DNA, 21 bp, artificial sequence
  synthetic oligonucleotide
gtatgtttgcgagcaagaaca

SEQ ID NO: 173 - DNA, 19 bp, artificial sequence
  synthetic oligonucleotide
ccaggtggaacctcatcag

SEQ ID NO: 174 - DNA, 21 bp, artificial sequence
  synthetic oligonucleotide
gcttagaattatggcctcact

SEQ ID NO: 175 - DNA, 22 bp, artificial sequence
  synthetic oligonucleotide
aacggtgtgacaagctacaaca

SEQ ID NO: 176 - DNA, 18 bp, artificial sequence
  synthetic oligonucleotide
aagcagttgtggcatctc

SEQ ID NO: 177 - DNA, 21 bp, artificial sequence
  synthetic oligonucleotide
gtcatgtgtggcggttcacta

SEQ ID NO: 178 - DNA, 179 bp, artificial sequence
  synthetic oligonucleotide
gcttagaattatggcctcacttgttcttgctcgcaaacatacaacgtgttgtagcttgtcacaccgtttctatagattagctaatgagtgtgctcaagtattgagtgaaatggtcatgtgtggcggttcactatatgttaaaccaggtggaacctcatcaggagatgccacaactgctt

SEQ ID NO: 179 - DNA, 21 bp, artificial sequence
  synthetic oligonucleotide
ccttatgggttgggattatcc

SEQ ID NO: 180 - DNA, 18 bp, artificial sequence
  synthetic oligonucleotide
tgtggcatctcctgatga

SEQ ID NO: 181 - DNA, 42 bp, artificial sequence
  synthetic oligonucleotide
cacgttgtatgtttgcgagcaagtgatagagccatgcctaac

SEQ ID NO: 182 - DNA, 42 bp, artificial sequence
  synthetic oligonucleotide
tgtagcttgtcacaccgtttctccacacatgaccatttcact

SEQ ID NO: 183 - DNA, 22 bp, artificial sequence
  synthetic oligonucleotide
agtgaggccataattctaagca

SEQ ID NO: 184 - DNA, 21 bp, artificial sequence
  synthetic oligonucleotide
agctaatgagtgtgctcaagt

SEQ ID NO: 185 - DNA, 20 bp, artificial sequence
  synthetic oligonucleotide
gtgatagagccatgcctaac

SEQ ID NO: 186 - DNA, 22 bp, artificial sequence
  synthetic oligonucleotide
cacgttgtatgtttgcgagcaa

SEQ ID NO: 187 - DNA, 20 bp, artificial sequence
  synthetic oligonucleotide
ccacacatgaccatttcact

SEQ ID NO: 188 - DNA, 22 bp, artificial sequence
  synthetic oligonucleotide
tgtagcttgtcacaccgtttct

SEQ ID NO: 189 - DNA, 145 bp, artificial sequence
  synthetic oligonucleotide
gtgatagagccatgcctaacatgcttagaattatggcctcacttgttcttgctcgcaaacatacaacgtgttgtagcttgtcacaccgtttctatagattagctaatgagtgtgctcaagtattgagtgaaatggtcatgtgtgg

SEQ ID NO: 190 - DNA, 21 bp, artificial sequence
  synthetic oligonucleotide
ccttatgggttgggattatcc

SEQ ID NO: 191 - DNA, 18 bp, artificial sequence
  synthetic oligonucleotide
tgtggcatctcctgatga

SEQ ID NO: 192 - DNA, 41 bp, artificial sequence
  synthetic oligonucleotide
cacgttgtatgtttgcgagcaaaatgtgatagagccatgcc

SEQ ID NO: 193 - DNA, 42 bp, artificial sequence; identical to SEQ ID NO: 182
  synthetic oligonucleotide

SEQ ID NO: 194 - DNA, 22 bp, artificial sequence
  synthetic oligonucleotide
agtgaggccataattctaagca

SEQ ID NO: 195 - DNA, 21 bp, artificial sequence
  synthetic oligonucleotide
agctaatgagtgtgctcaagt

SEQ ID NO: 196 - DNA, 19 bp, artificial sequence
  synthetic oligonucleotide
aatgtgatagagccatgcc

SEQ ID NO: 197 - DNA, 22 bp, artificial sequence
  synthetic oligonucleotide
cacgttgtatgtttgcgagcaa

SEQ ID NO: 198 - DNA, 20 bp, artificial sequence
  synthetic oligonucleotide
ccacacatgaccatttcact

SEQ ID NO: 199 - DNA, 22 bp, artificial sequence
  synthetic oligonucleotide
tgtagcttgtcacaccgtttct

SEQ ID NO: 200 - DNA, 148 bp, artificial sequence
  synthetic oligonucleotide
aatgtgatagagccatgcctaacatgcttagaattatggcctcacttgttcttgctcgcaaacatacaacgtgttgtagcttgtcacaccgtttctatagattagctaatgagtgtgctcaagtattgagtgaaatggtcatgtgtgg

SEQ ID NO: 201 - DNA, 21 bp, artificial sequence
  synthetic oligonucleotide
ccttatgggttgggattatcc

SEQ ID NO: 202 - DNA, 18 bp, artificial sequence
  synthetic oligonucleotide
tgtggcatctcctgatga

SEQ ID NO: 203 - DNA, 42 bp, artificial sequence
  synthetic oligonucleotide
cacgttgtatgtttgcgagcaaatgtgatagagccatgccta

SEQ ID NO: 204 - DNA, 42 bp, artificial sequence; identical to SEQ ID NO: 182
  synthetic oligonucleotide

SEQ ID NO: 205 - DNA, 22 bp, artificial sequence
  synthetic oligonucleotide
agtgaggccataattctaagca

SEQ ID NO: 206 - DNA, 21 bp, artificial sequence
  synthetic oligonucleotide
agctaatgagtgtgctcaagt

SEQ ID NO: 207 - DNA, 20 bp, artificial sequence
  synthetic oligonucleotide
atgtgatagagccatgccta

SEQ ID NO: 208 - DNA, 22 bp, artificial sequence
  synthetic oligonucleotide
cacgttgtatgtttgcgagcaa

SEQ ID NO: 209 - DNA, 20 bp, artificial sequence
  synthetic oligonucleotide
ccacacatgaccatttcact

SEQ ID NO: 210 - DNA, 22 bp, artificial sequence
  synthetic oligonucleotide
tgtagcttgtcacaccgtttct

SEQ ID NO: 211 - DNA, 147 bp, artificial sequence
  synthetic oligonucleotide
atgtgatagagccatgcctaacatgcttagaattatggcctcacttgttcttgctcgcaaacatacaacgtgttgtagcttgtcacaccgtttctatagattagctaatgagtgtgctcaagtattgagtgaaatggtcatgtgtgg

SEQ ID NO: 212 - DNA, 22 bp, artificial sequence
  synthetic oligonucleotide
cacagttacttcacttcagact

SEQ ID NO: 213 - DNA, 18 bp, artificial sequence
  synthetic oligonucleotide
cgcagtaaggatggctag

SEQ ID NO: 214 - DNA, 41 bp, artificial sequence
  synthetic oligonucleotide
gctagtagtcgtcgtcggttctgatgagcctgaagaacatg

SEQ ID NO: 215 - DNA, 44 bp, artificial sequence
  synthetic oligonucleotide
aagcacaagctgatgagtacgagtaactagcaagaataccacga

SEQ ID NO: 216 - DNA, 20 bp, artificial sequence
  synthetic oligonucleotide
ggatgaaccgtcgattgtgt

SEQ ID NO: 217 - DNA, 19 bp, artificial sequence
  synthetic oligonucleotide
ttcggaagagacaggtacg

SEQ ID NO: 218 - DNA, 20 bp, artificial sequence
  synthetic oligonucleotide
tgatgagcctgaagaacatg

SEQ ID NO: 219 - DNA, 21 bp, artificial sequence
  synthetic oligonucleotide
gctagtagtcgtcgtcggttc

SEQ ID NO: 220 - DNA, 22 bp, artificial sequence
  synthetic oligonucleotide
gtaactagcaagaataccacga

SEQ ID NO: 221 - DNA, 22 bp, artificial sequence
  synthetic oligonucleotide
aagcacaagctgatgagtacga

SEQ ID NO: 222 - DNA, 231 bp, artificial sequence
  synthetic oligonucleotide
tgatgagcctgaagaacatgtccaaattcacacaatcgacggttcatccggagttgttaatccagtaatggaaccaatttatgatgaaccgacgacgactactagcgtgcctttgtaagcacaagctgatgagtacgaacttatgtactcattcgtttcggaagagacaggtacgttaatagttaatagcgtacttctttttcttgctttcgtggtattcttgctagttac

SEQ ID NO: 223 - DNA, 20 bp, artificial sequence
  synthetic oligonucleotide
agttccttgttgtaacggtt

SEQ ID NO: 224 - DNA, 20 bp, artificial sequence
  synthetic oligonucleotide
ctgctgaggcttctaagaag

SEQ ID NO: 225 - DNA, 10 bp, artificial sequence
  synthetic oligonucleotide
acaagctaca

SEQ ID NO: 226 - DNA, 10 bp, artificial sequence
  synthetic oligonucleotide
atacaacgtg